European Patent Application EP 4 309 662 A1, published January 24, 2024. Title: MICROORGANISMS CONVERTING INOSITOL TO BUTYRATE. Applicant: Enbiosis Biotechnology Limited. The sequence listing filed with the application follows.

SEQUENCE LISTING (28 sequences)

SEQ ID NO: 1 - DNA, 1143 bp, synthetic construct
  source 1..1143: mol_type = other DNA
atggttgaatttaaattaacgaaagaacaactgcttgcaaaggaattgttcagaagtttcgctgagaatgagatcaaaccaatttccagagatatggatgaagcagagaaatttgatatggatctgttagataagatgaagaaatacggtctgatgggaattccatattctaaagaatacggtggagagggagcagatgtattaacatatgctttagcaatggaagaggtatccaaagttgatgccagtgcaggaatcacaatttccgtacatacttctctttgctgttcttgtattaacgactatgcatcagaagaacagaaacagaaattcttacgtccattagttgacggaagtaagattggatgttttggactgacagaaccaggagctggaacagatgccagcggagttaaaacaactgcaaaattagacggtgatcattatgtattaaatggtcagaaagtatttacaacaaactctggatttgcagatacattcattatttttgcttacacagataagagtgcaggaacaagaggtatgtctgcatttatcgtagatagagacagcgaaggattaacagtcagcaaagatattcctcgtatgggaatcagagcagcatccaacgcagaagtagcattagttgatgtgaaagttccaaaagaaaacctgatcggaagagaaggaatgggatataagatcgctatgggagctttaacaggaggacgtatcggaatcggtgctcagtctgttggtattgcacagggtgcattaaatgaagcaatcaaatacgtaaaagaaagaaaacagtttggaaaaccaatagcaaaattccagaatacacagttcttgatcgcagcattacagacaaagattgatgcagcaagattaatggtatggagagcagcgaaagcaaaagatgatcatgaaaattttgcaccacttgcagcacagtgtaaattatttgcttctgatgtagctgttgaagttacaagaggagcagttcagatgcttggtggatatggatactcaagagaatatccagtagagagaatgtatcgtgatgcaaagatcacagagatttatgaaggtacatccgaagctatgaagatgatcgttggcggtggattattaagataa

SEQ ID NO: 2 - protein, 380 aa, synthetic construct
MVEFKLTKEQLLAKELFRSFAENEIKPISRDMDEAEKFDMDLLDKMKKYGLMGIPYSKEYGGEGADVLTYALAMEEVSKVDASAGITISVHTSLCCSCINDYASEEQKQKFLRPLVDGSKIGCFGLTEPGAGTDASGVKTTAKLDGDHYVLNGQKVFTTNSGFADTFIIFAYTDKSAGTRGMSAFIVDRDSEGLTVSKDIPRMGIRAASNAEVALVDVKVPKENLIGREGMGYKIAMGALTGGRIGIGAQSVGIAQGALNEAIKYVKERKQFGKPIAKFQNTQFLIAALQTKIDAARLMVWRAAKAKDDHENFAPLAAQCKLFASDVAVEVTRGAVQMLGGYGYSREYPVERMYRDAKITEIYEGTSEAMKMIVGGGLLR

SEQ ID NO: 3 - DNA, 798 bp, synthetic construct
  source 1..798: mol_type = other DNA
atgaagattgttgtttgtgcaaaacaagtaccagatacaacggaagtaaaattagatccaaagacaaatacactgatccgtgatggtgttccaagtattattaacccagatgataaagcaggaattgaagcagcacttcagttaaaagaaaaatgcccaggaagtacagtaactgttgtttctatgggaccacctcaggcagatgttgcattaagagaagcattagcaatgggatgcgatgatgcattattgatctcagatcgtgcatttggaggagcagatacatgggctacttcttctacaattgcagcagcattaaagaaattagactatgatgtgatcatcacaggtcgtcaggcaatcgatggagatacagcgcaggttggaccgcagatcgcagaacaccttggaatccctcaggtaagttatgtagagaagatggatgtagaaggggaagatactttagttgtccagagacagtttgaagatcgtcaccagatcatcgaggtgaagacaccttgtcttttaacagcattagctgaacttgctgatccaagatatatgtctgttcacggtgtatttgatgcatatcgtgaaaaagaagttaaagtatggggattagaagatatcaaagatacagtcaatgaaggaaatatcggattaaaaggttctcctaccagagttaagaaatcctttacaaaacaggcaaaaggtgcaggaacgatcttaaatgatctctccgatgacgaagcagttgccgcaatcgtagaaaaattacaggaaaaacacatcatttaa

SEQ ID NO: 4 - protein, 265 aa, synthetic construct
MKIVVCAKQVPDTTEVKLDPKTNTLIRDGVPSIINPDDKAGIEAALQLKEKCPGSTVTVVSMGPPQADVALREALAMGCDDALLISDRAFGGADTWATSSTIAAALKKLDYDVIITGRQAIDGDTAQVGPQIAEHLGIPQVSYVEKMDVEGEDTLVVQRQFEDRHQIIEVKTPCLLTALAELADPRYMSVHGVFDAYREKEVKVWGLEDIKDTVNEGNIGLKGSPTRVKKSFTKQAKGAGTILNDLSDDEAVAAIVEKLQEKHII

SEQ ID NO: 5 - DNA, 996 bp, synthetic construct
  source 1..996: mol_type = other DNA
atgtgtaaagatgtttatgtatttgctgagcagagagatggaaatcttcagaaagtcggtatcgaactgatcggagaagcaagaaagcttgcagatgatcttggacagaatgtagttgcagttttacttggaaatcagattaaagacaaagcaagtgaactgatcgctcatggagcagataaagttgtagtagtagatgatgaaatgctggcagaatatgtgacagaaccatatgcaaaagcaatgatggagatcattcagtcccataatccagagattgttctctatggagcaacatcgatcggacgagatcttgcaccaagagtttctgcaagaatccacacaggattaacagcagactgtacaaaacttgatattgatgaagaaacaaaattattaatgatgacacgaccagcatttggtggaaatatcatggctacgatcgtctgtgaagatttcagaccacagatggcaacggtaagacctggtgttatgaaagcattagaagctgatgaaagcagacaaggtgaggttgaagttgttgaagtaaactttacagatgcagatatgaatgttaagatccgtgaagttgtaaaaacaacacacaaatctgtagatatcacagaagctaagatcctggtagcaggaggacgtggtgtaggaaatgcagaaggatttaaagatcttgaagcattagcggatacattagatggtgaagtggcagcatcaagagcagctgtagattcaggatggatcagcaatgaccgtcaggttggacagacaggtaagacggttcgtccagagttatacttagcatgtggaatttctggagcgatccagcacgcagcaggtatggagaattcagaattcatcgtagcgatcaaccgagatgaagacgcagcgatctttgatatcgcagatcttggtgtcgtgggtgatattaagaagatccttccaaaattaaatgatgcgatcaaagcagtcaaagaaaaataa

SEQ ID NO: 6 - protein, 331 aa, synthetic construct
MCKDVYVFAEQRDGNLQKVGIELIGEARKLADDLGQNVVAVLLGNQIKDKASELIAHGADKVVVVDDEMLAEYVTEPYAKAMMEIIQSHNPEIVLYGATSIGRDLAPRVSARIHTGLTADCTKLDIDEETKLLMMTRPAFGGNIMATIVCEDFRPQMATVRPGVMKALEADESRQGEVEVVEVNFTDADMNVKIREVVKTTHKSVDITEAKILVAGGRGVGNAEGFKDLEALADTLDGEVAASRAAVDSGWISNDRQVGQTGKTVRPELYLACGISGAIQHAAGMENSEFIVAINRDEDAAIFDIADLGVVGDIKKILPKLNDAIKAVKEK

SEQ ID NO: 7 - DNA, 759 bp, synthetic construct
  source 1..759: mol_type = other DNA
atgagatttgttgtgattttaaaacaaattccagatgattcgatcaaaaaagaatatcaggatgtggatcagttaaatgacagtgataagaacgtaataaaagaagcactggatttaagagaccgctatggtggaactgtagatgtgatcggatttggaccattatctgcagaagatgttatgaaagagacgcttacttatggaattgatgatgccttcctgatcagtgattcccaattcgcagatatggatgtatcacaggtagccaagatcgtcgcagcggtgatcaaaaagcttggtccatatgatctggtcttatgcggacggcaggcaattgatggagatagtgcccatatggcttctatgacctcttgtgcgttggagatcccattgatcgcgtattctgacgagatcacagagatgaaagatggaagtgttttcgcaacatgtatgggtgatcagatggcatataaggtagaagcaaaaactccagcaatgatactttctatcagagagaagaacaagaaccgttttccatccgtaccagatatcatgaaaacatatgatggaacatataagacaaagatattgacgaatgaagacctgaatttttctgtgaccaagagaaaagtaacgcaacttagaaaatatgaagtcaaaagcagcaaacagcaaaaacttgttatgatcggtggaaaagacgaagaagaaaaagcggcacagattcttcagttattaaagcaaaagagcgtgatctag

SEQ ID NO: 8 - protein, 252 aa, synthetic construct
MRFVVILKQIPDDSIKKEYQDVDQLNDSDKNVIKEALDLRDRYGGTVDVIGFGPLSAEDVMKETLTYGIDDAFLISDSQFADMDVSQVAKIVAAVIKKLGPYDLVLCGRQAIDGDSAHMASMTSCALEIPLIAYSDEITEMKDGSVFATCMGDQMAYKVEAKTPAMILSIREKNKNRFPSVPDIMKTYDGTYKTKILTNEDLNFSVTKRKVTQLRKYEVKSSKQQKLVMIGGKDEEEKAAQILQLLKQKSVI

SEQ ID NO: 9 - DNA, 1011 bp, synthetic construct
  source 1..1011: mol_type = other DNA
atgaatttagggaaaaaagaaggaatcgttgttgttggagagattcaaaagagagagatcatgccgctgacgttggaattgatcggggcagcaggaaaactttcgaaggaaagagatctttcattgtcagttattctatcagaatgtgggatcaaagaagaggcaaagaagctttacaattacggagttgatgaaatcctctgtatcgaagatgaaaaattaatagaaggacatatgcagctgcatcatgatgctgtcatagaagttttaaaaggaaaggatccgaaagtgatactgatcggaggaacagcatcaggaagagttcttgcaggaaagacagcttatgcatttgatacagaattagtctgtgatgcatcgaaacttacatacgatgagaaacaggaacaacttatcatcacaagaccggcattcgatggaaaaaatatggcagactttgtgatcaatccatccttgacatcggtgatcacgatccgtacaggagtgatgggaaaagcagaatacaaggaagacaaacaaggtgagatgttatatgtatatccagaatgtctgaaggaagaacgacaagatctgatctatcacggagtggcaggaaaaagtggaaaagaagttcatctggatacagcaaggatcatagtttccggtggccgtgggatgaaaggagaagaaggatttgcgcttcttgagagacttgcagagaagatcggaggggaagttgcatgtacaagaccatgtgtagatgccggatggatgcttccaacacagcaggtaggacagtcaggaatctccgtaaaaccgaaactgtatcttgcatttgggattgccggggcaattcagcatatgacaggaattgatgcagattgcatcatttcagtcaataataatccgagggctgcgatctttgcatacagtgattatggtgtggtttcggatgcaaagaaattactggagagtatgttaaaacagatggaagaaggaaaagaattcttataa

SEQ ID NO: 10 - protein, 336 aa, synthetic construct
MNLGKKEGIVVVGEIQKREIMPLTLELIGAAGKLSKERDLSLSVILSECGIKEEAKKLYNYGVDEILCIEDEKLIEGHMQLHHDAVIEVLKGKDPKVILIGGTASGRVLAGKTAYAFDTELVCDASKLTYDEKQEQLIITRPAFDGKNMADFVINPSLTSVITIRTGVMGKAEYKEDKQGEMLYVYPECLKEERQDLIYHGVAGKSGKEVHLDTARIIVSGGRGMKGEEGFALLERLAEKIGGEVACTRPCVDAGWMLPTQQVGQSGISVKPKLYLAFGIAGAIQHMTGIDADCIISVNNNPRAAIFAYSDYGVVSDAKKLLESMLKQMEEGKEFL

SEQ ID NO: 11 - DNA, 1596 bp, synthetic construct
  source 1..1596: mol_type = other DNA
atgaaacctgtaaaaccacctcgtattaatggacgagtgccggtcctgtcggcacaggaagcggtgaattatattcccgacgaagcaacactttgtgtgttaggcgctggcggcggtattctggaagccaccacgttaattactgctcttgctgataaatataaacagactcaaacaccacgtaatttatcgattattagtccaacagggcttggcgatcgcgccgaccgtggtattagtcctctggcgcaagaaggtctggtgaaatgggcattatgtggtcactggggacaatcgccgcgtatttctgaactcgcagaacaaaataaaattattgcttataactacccacaaggtgtacttacacaaaccttacgcgccgccgcagcccaccagcctggtattattagtgatattggcatcgggacatttgtcgatccacgccagcaaggcggcaaactgaatgaagtcactaaagaagacctgattaaactggtcgagtttgataacaaagaatatctctattacaaagcgattgcgccagatattgccttcattcgcgctaccacctgcgacagtgaaggctacgccacttttgaagatgaggtgatgtatctcgacgcattggttattgcccaggcggtgcacaataacggcggtattgtgatgatgcaggtgcagaaaatggttaagaaagccacgctgcatcctaaatctgtccgtattccgggttatctggtggatattgtggtggtcgatccggatcaaacccaactgtatggcggtgcaccggttaaccgctttatttctggtgacttcacccttgatgacagtaccaaacttagcctgcccctaaaccaacgtaaattagttgcgcggcgcgcattattcgaaatgcgtaaaggcgcggtggggaatgtcggcgtcggtattgctgacggcattggcctggtcgcccgagaagaaggttgtgctgatgactttattctgacggtagaaacaggtccgattggcggaattacttcacaggggatcgcctttggcgcgaacgtgaatacccgtgccattctggatatgacgtcccagtttgatttttatcacggtggcggtctggatgtttgttatttgagttttgctgaagtcgaccagcacggtaacgtcggcgtgcataaattcaatggtaaaatcatgggcaccggtggatttattgatatcagtgccacttcgaagaaaatcattttctgcggcacattaactgcgggcagtttaaaaacagaaattaccgacggcaaattaaatatcgtccaggaaggacgggtgaagaaatttattcgggaactaccggaaattactttcagcggaaaaatcgctctcgagcgagggctggatgttcgttatatcactgagcgcgcagtattcacgctgaaagaagacggcctgcatttaatcgaaatcgcccctggcgtcgatttacaaaaagatattctcgacaaaatggatttcaccccagtgatttcgccagaactcaaactgatggacgaaagattatttatcgatgcggcgatgggttttgtcctgcctgaagcggctcattaa

SEQ ID NO: 12 - protein, 531 aa, synthetic construct
MKPVKPPRINGRVPVLSAQEAVNYIPDEATLCVLGAGGGILEATTLITALADKYKQTQTPRNLSIISPTGLGDRADRGISPLAQEGLVKWALCGHWGQSPRISELAEQNKIIAYNYPQGVLTQTLRAAAAHQPGIISDIGIGTFVDPRQQGGKLNEVTKEDLIKLVEFDNKEYLYYKAIAPDIAFIRATTCDSEGYATFEDEVMYLDALVIAQAVHNNGGIVMMQVQKMVKKATLHPKSVRIPGYLVDIVVVDPDQTQLYGGAPVNRFISGDFTLDDSTKLSLPLNQRKLVARRALFEMRKGAVGNVGVGIADGIGLVAREEGCADDFILTVETGPIGGITSQGIAFGANVNTRAILDMTSQFDFYHGGGLDVCYLSFAEVDQHGNVGVHKFNGKIMGTGGFIDISATSKKIIFCGTLTAGSLKTEITDGKLNIVQEGRVKKFIRELPEITFSGKIALERGLDVRYITERAVFTLKEDGLHLIEIAPGVDLQKDILDKMDFTPVISPELKLMDERLFIDAAMGFVLPEAAH

SEQ ID NO: 13 - DNA, 777 bp, synthetic construct
  source 1..777: mol_type = other DNA
atgaacaatttattaatggaagtggaaaacgaaatcgccgttgttactattaaccgtccaaaatctttaaacgccctaaacagtgaaactttagcagaacttgatgcttgcttctctgaaatttctgagagaaaagatatcaaagttgtgatcttaacaggttctggagcaaaagctttcgttgctggagctgatatctctgaaatggtaaatgcaacacctgcagaaggtagaaaaatgggaatgcttgcaaaagaagctttcttaaaacttgaaacaatgcctcaggttacgatcgctgctgtcaatggtttcgcattaggtggtgggtgtgagatctctatggcttgtgatatccgtatcgcatctgataacgcaaaattcggacagcctgaaacaggacttggtatccttcctggtttcggtggaacacagcgtcttgctcgtctggttggtaaaggacgtgcaaaagaattgatctttacatgtgatatgatcgatgctaatgaagcttacagaatcggacttgctaacaaagtagttcctcaggctgaattacttgatacctgtaaggcaatggctgagaagatcatgagcaaaggaagctatgctatttctcttgcaaaagaagcaatcaacactggtacagaaacagacctttcaagcggattaacattagaagcagacttatttggtcttgcattctcaactgatgacaaaaaagaaggtatgacagctttcttagagaaacgtaaagcaaatcttacagatttctag

SEQ ID NO: 14 - protein, 258 aa, synthetic construct
MNNLLMEVENEIAVVTINRPKSLNALNSETLAELDACFSEISERKDIKVVILTGSGAKAFVAGADISEMVNATPAEGRKMGMLAKEAFLKLETMPQVTIAAVNGFALGGGCEISMACDIRIASDNAKFGQPETGLGILPGFGGTQRLARLVGKGRAKELIFTCDMIDANEAYRIGLANKVVPQAELLDTCKAMAEKIMSKGSYAISLAKEAINTGTETDLSSGLTLEADLFGLAFSTDDKKEGMTAFLEKRKANLTDF

SEQ ID NO: 15 - DNA, 1014 bp, synthetic construct
  source 1..1014: mol_type = other DNA
atggtaaacgtaggaattattggagcaggaagaatcggacaggtacacatgaacagcattttaacaagagtaccaaatgcaaagatcaaagcagttgcagatccattcttaagtgaagaagcagacaagaaagcaaaagcagctggagcagagtatacaacaaaagattacaaagatatcttagcagacaaagatattgatgcagtgatcatttgttcatcaacagatactcattccccaatctcaattgaagcgatcaaagcaggaaaacatgtattttgtgaaaaaccgatcgatcatgatgtagacaagatcaaagaagttatcaaaacattagaaggaacaggacttaaatatcaggtaggatttaacagaagatttgaccacaactttgaagcagcacagagagctgttgtcaatggaaagatcggagcacctcatatcatcaagatcacatcaagagatcctgagccaccaagtgctgaatatgtaaaagtatctggaggaatgttccttgatatgacaattcatgattttgatatggtacgattccttgcaggatgtgatgcagaagaagtttatgtacaggcagcaaaccttgtagatcctgagattggaaaagcaggtgatgttgacacagcgatcatcacattgaagatggaaaatggagcacttgcagtaatcgataactctcgtcaggcagtttatggatatgatcagagagcagaagtattcggatctaaaggaatggtagcgatcaagaatgattctgattctacagcagtgatcagcaacgaagatggtgtaacaggagaaaaaccacagttcttcttccttgaaagatacatggatgcatatggaaaagaaatggttcagttcattgatgcaattgaaaatgacacagaaacaccattaggagtagaagatggattaaaaccagtacttatgggacttgcagcaaagaaatcagtagaagaaggccgtccagtaaaaatttcagaaattgaattctaa

SEQ ID NO: 16 - protein, 337 aa, synthetic construct
MVNVGIIGAGRIGQVHMNSILTRVPNAKIKAVADPFLSEEADKKAKAAGAEYTTKDYKDILADKDIDAVIICSSTDTHSPISIEAIKAGKHVFCEKPIDHDVDKIKEVIKTLEGTGLKYQVGFNRRFDHNFEAAQRAVVNGKIGAPHIIKITSRDPEPPSAEYVKVSGGMFLDMTIHDFDMVRFLAGCDAEEVYVQAANLVDPEIGKAGDVDTAIITLKMENGALAVIDNSRQAVYGYDQRAEVFGSKGMVAIKNDSDSTAVISNEDGVTGEKPQFFFLERYMDAYGKEMVQFIDAIENDTETPLGVEDGLKPVLMGLAAKKSVEEGRPVKISEIEF

SEQ ID NO: 17 - DNA, 900 bp, synthetic construct
  source 1..900: mol_type = other DNA
atgtttgataagaataaagtaaaattaggaattgcaccaatcgcatggacaaatgatgatcttccagatcttggagctgaaaatacatttgaacagtgtgtcagtgaaatggcacttgcaggatttacagggtcagaagtaggaaataaatatccaaaagatccagcagaattaaagaaagcattagatcttcgtggaatcgaaatttgtaatcagtggttttcatctttcctgatcacaaaaccattagaggaagtagaaaaagaattccgtgcacagttagagttcttaaaagcaatgggagcaaaagtgatcggagcttctgaacaaagttacagtgtacagggacaggaagatacaccagtttttggacataaatatgtgatggacgatgaagaatgggatacattctgcaacggaatgaattatcttggaaagattgcaaaagaggaatacggaatcgcattaacattccatcatcatatgggaacagtcgtacaagacccagatgaagtagaacgcatgatggcaaatacagatccagaatacgtaagtttattattcgatacaggacattttacttactgtggagcagatccattagaaatggtgaaaaaatatgtaaaccgtattaaacatgtgcatttaaaagatatccgtccagaagttgtaaaagaagtgaaagacaacgatttaagcttccttgaaggagtaagaagaggtgcatttacagtacctggagatggatgtattgattttgatccgatctttaaagtattagaggagaatggatatgaaggatatatgcttgtagaagcagaacaagatccagcaaaagcaaatccattagaatatgcgatcaaagcacgtaaatttatcagagaaaaaactggattataa

SEQ ID NO: 18 - protein, 299 aa, synthetic construct
MFDKNKVKLGIAPIAWTNDDLPDLGAENTFEQCVSEMALAGFTGSEVGNKYPKDPAELKKALDLRGIEICNQWFSSFLITKPLEEVEKEFRAQLEFLKAMGAKVIGASEQSYSVQGQEDTPVFGHKYVMDDEEWDTFCNGMNYLGKIAKEEYGIALTFHHHMGTVVQDPDEVERMMANTDPEYVSLLFDTGHFTYCGADPLEMVKKYVNRIKHVHLKDIRPEVVKEVKDNDLSFLEGVRRGAFTVPGDGCIDFDPIFKVLEENGYEGYMLVEAEQDPAKANPLEYAIKARKFIREKTGL

SEQ ID NO: 19 - DNA, 933 bp, synthetic construct
  source 1..933: mol_type = other DNA
atgaaggattcatattttgaaaggcaaaaggtgaaggatatgttagataagaaaaaagtaaaattaggaattgctccaattggatggacaaacgatgatatgccagatcttggaaaagaaaatacctttcagcagtgtgtgagtgaaatggcattggctggatttacaggatctgaagtagggggaaaatatcctacagatgtagaaacactaaaaaaggcattagatttaagaggaatacagatctgtaactgttggttttctagtttcttgatttccagaccatatgaagaaaccgaaaaagaatttatcaaacagacagatttcttaaaggcaatgggagcaaaagtcattggagtatctgagcaaagttatagcattcagggcaaagaccagccgatctttgaaggaaaatatgtaatgaatgatgaggaatggaaactgctcacagatgggttaaataaacttggacagattgcaaaagacaaaggaatgatgttaacattccatcatcatatgggaacagtgatacagacagaagaagaaatcgatcgttttatgaacgaagttgataaagacctggtttatctgttatttgatagtggacattgctcatttgctgggattgatccagtcaaagttttaagcaaatatattgaccgtacaagacatatccatttaaaagatttaagatctgatgttgtagcacagtcaaagaaagaaggctggagtttcttaaaaggtgtcagagaaggaacatttacagttccaggagatggagatgtagattttgcaccaatttttgatatcatcgaaaaaagtggatatgaaggatatgttgtggtagaagcagaacaagatccagcaaaagccaatccattagaatatgcaatgaaagcaagaaaatatattgcagagaaaacaggattataa

SEQ ID NO: 20 - protein, 310 aa, synthetic construct
MKDSYFERQKVKDMLDKKKVKLGIAPIGWTNDDMPDLGKENTFQQCVSEMALAGFTGSEVGGKYPTDVETLKKALDLRGIQICNCWFSSFLISRPYEETEKEFIKQTDFLKAMGAKVIGVSEQSYSIQGKDQPIFEGKYVMNDEEWKLLTDGLNKLGQIAKDKGMMLTFHHHMGTVIQTEEEIDRFMNEVDKDLVYLLFDSGHCSFAGIDPVKVLSKYIDRTRHIHLKDLRSDVVAQSKKEGWSFLKGVREGTFTVPGDGDVDFAPIFDIIEKSGYEGYVVVEAEQDPAKANPLEYAMKARKYIAEKTGL

SEQ ID NO: 21 - DNA, 1023 bp, synthetic construct
  source 1..1023: mol_type = other DNA
atgagatatgtagaatttgatgaaacaagacctatggatttaattttattaggacgtgtcgctattgattttaatccatcagaagatgagccattcggaccacttgagaatgtcagaacttttaagaagtatgttggtggttctccagcaaatatcgcagttggggttacaagacatggattaaaagcaggatttcttgggaaagtatctgatgataagtttggtaaattcgtagttgactttttcaataaagaaggaattgatacaagtcatattacaaaatgtacaaacggtgaaaaactaggacttacatttacagagatgctatcagaaaaagaaagcagcatcctgatgtatcgaaattgcatcgcagacttacagttatctgtcgatgacattgatgaagattacatcaaacagtcaaaagcaatcctgatctcaggaacagcacttgcagaaagcccatcaagagaagcagctttaaaagcagtgatgttagcaaagaaaaatgatacaaagatcatttttgatattgattatagagaatataactggaagagtgaagatgaaatctctatttactattctatggtagcaagagaagcagatatcatcatgggatccagagaagagtttgacttaacagagaaactgatccagccaggaagaacagatgaagaaacagcagctgcatggcatgcatacaatgcgaagatcgttgttatcaaacatggtatgaaaggatctacagcatacacgattgatggacagaacttctcaatcaaaccattcccagtcaatgcaagaaaaggattcggtggaggagatggttatggatcagccttcttatatggaatctatcagggatgggaagttatcgactgtttagagttcggatcagcagaagcatctatgatggtaagaagtaattcttgttccgaagaacttccaaacccacagcaggtaaaagacttcattaaagaaacaaaagaaaaatacggagaaatgatcgcaagagtatag

SEQ ID NO: 22 - protein, 340 aa, synthetic construct
MRYVEFDETRPMDLILLGRVAIDFNPSEDEPFGPLENVRTFKKYVGGSPANIAVGVTRHGLKAGFLGKVSDDKFGKFVVDFFNKEGIDTSHITKCTNGEKLGLTFTEMLSEKESSILMYRNCIADLQLSVDDIDEDYIKQSKAILISGTALAESPSREAALKAVMLAKKNDTKIIFDIDYREYNWKSEDEISIYYSMVAREADIIMGSREEFDLTEKLIQPGRTDEETAAAWHAYNAKIVVIKHGMKGSTAYTIDGQNFSIKPFPVNARKGFGGGDGYGSAFLYGIYQGWEVIDCLEFGSAEASMMVRSNSCSEELPNPQQVKDFIKETKEKYGEMIARV

SEQ ID NO: 23 - DNA, 1929 bp, synthetic construct
  source 1..1929: mol_type = other DNA
atggcaaagacagtaagaatgacagttgctcaggcaattgtaaagtttttagataatcagtatgtttcaatggacggagaagaaacaaaatttgtagaaggattcttcacaatcttcggacatggaatcgcagttggacttggagaagcacttgataccaatccaggaaacttaagagttcttcagggaagaaatgaacagggaatgtgtcatgttgcaacagcttatgcaaaacagaatggaagaaagaagatcattccttgtgcatcatctgtaggacctggagctgcgaatatggtaacagcttgtgcgacagctacagtgaataatattccattattagtatttccagcagatacatttgcatcaagacagccagacccagttcttcagcagttagagcagagcaatagtttatcaacaacaacaaatgatgcatttaagccagtgtgcaaatattgggaccgagttacaagaccagaacatatcatgacagcactgatcaatgcaatgagagttttaacagatccagcagaaacaggagcatgctgcatcggtctttgccaggatgttgaaggtgaatcttttgatttccctgaatatttctttgagaaacgagttcacaggatcacaagaccagtggcagtggaagaagagattgaagacattgcaaatgtgatcgcaaatgcgaagaaaccacttgttatcgttggtggaggtgttcgttactctgaagctggggaagaagtagaaaaattttgtgaagaattcaagattccatttggtgagacacagggaggaaaaagtgcatgtagatcaagccatccatactgcatgggaggaatcggtgttacaggtacttatgcatccaatgttcttgcaaaagatgcggatgtagtcattgcaatcggaagcagaatgtcagatttcgcgacaggatccaagagacagtttgcaaatcctgatgtgaagtttgtatctatcaataacagcagatatcatgcatataaattagattctgtgaaagcagttggagatgcaaaagtaacagtgaaagcattagctgaaaaattaagagcaatgaattatgtttcatcttataatggagagattgaagaagccaaggctgtatgggataaagaaatgaaacgtctggctgagtacaaatatgatgaaacatttgaaccaatgatcaaaaatatggatccaagaacaattccagaattcgtggagctgacaaaaggtaagatcacacagacagcagcattagcaacgatcagagatgtgatcgatgaagatgcaacgatcatcacagcaggaggaagcttaccaagttgtatgcagcgtgtatggacaacagataaacgtggtggatatcatgcagagtacggatattcttgtatgggatatgaagttgcagcagcactcggagttaaacttgcagagcctgacaatgaagtctatgcagttgttggagatgcaagtttccagatgttacacagtgagatcatgacaatgatgcaggaaaaacagaaagcaaatatcttagtattcgataactgtggatttggatgcatcaataatctgcagatgaatcatggtattggatcccttgcaacagaattccgttacagagaaggaaataaaccttgcggagatctgatcccagttgattatgcaaaagttgcagaaggatatggattaaaatcttatacatgtaagacgatcgaagaattaagagcagccttagaagatgctaagaaacaaaacgttgcatgcttatttgacttaaaagtaattccaaagacaatgacagatggatatgaatcatggtggaatgttggaattgctacaacttctgaaaaagaaagcgttcgcaaggcatgtgaaggtgttatggaaggaagaaaagaagcaagagcttactaa

SEQ ID NO: 24 - protein, 642 aa, synthetic construct
MAKTVRMTVAQAIVKFLDNQYVSMDGEETKFVEGFFTIFGHGIAVGLGEALDTNPGNLRVLQGRNEQGMCHVATAYAKQNGRKKIIPCASSVGPGAANMVTACATATVNNIPLLVFPADTFASRQPDPVLQQLEQSNSLSTTTNDAFKPVCKYWDRVTRPEHIMTALINAMRVLTDPAETGACCIGLCQDVEGESFDFPEYFFEKRVHRITRPVAVEEEIEDIANVIANAKKPLVIVGGGVRYSEAGEEVEKFCEEFKIPFGETQGGKSACRSSHPYCMGGIGVTGTYASNVLAKDADVVIAIGSRMSDFATGSKRQFANPDVKFVSINNSRYHAYKLDSVKAVGDAKVTVKALAEKLRAMNYVSSYNGEIEEAKAVWDKEMKRLAEYKYDETFEPMIKNMDPRTIPEFVELTKGKITQTAALATIRDVIDEDATIITAGGSLPSCMQRVWTTDKRGGYHAEYGYSCMGYEVAAALGVKLAEPDNEVYAVVGDASFQMLHSEIMTMMQEKQKANILVFDNCGFGCINNLQMNHGIGSLATEFRYREGNKPCGDLIPVDYAKVAEGYGLKSYTCKTIEELRAALEDAKKQNVACLFDLKVIPKTMTDGYESWWNVGIATTSEKESVRKACEGVMEGRKEARAY

SEQ ID NO: 25 - DNA, 786 bp, synthetic construct
  source 1..786: mol_type = other DNA
atgggtaaagtatttggatatcctgaatttgatgaaaatggagaacagatcttaacaacttatgacaatgaatataaggatatgttaatggatgttcgagtatatcgaatgaaggcaggagacgaaaaaagttttcaaaagacaggtgaggaaacagcagtcttattattaagcggttctattgaatttgtatttgatgatgtgacagcgaaagcagatcgaaaggatgttttcacagaaggaccttggtgtgtgcatgcagcaacagaatctaaggtaagtgttaaggcacttgcagatagtgagatccttgttcagtcaacaaagaatgatacaaagtttgacactaaattatataaaccagaagatgctccatggggatattcttctgttggtaaatttggaaatgtggcaaaacgccgtgtaaatacgatctttgatcatgatatcgctccatattctaatatggtacttggagaagtattaaatgacagaggaaactggtcaggatatctgccacacagacacccacagccagaaacttactactttaaatttgaccgtccggaaggatttggagcaagtttcgtaggtgatcaggtatttaaaagtacagatggaagtttttcagcaatcccaggtggagaattacatccacaggctgttgcaccaggattccagatgtatacatgctggatgatccgccatctggatggaaacccttggttacagacagatcgaaatgaagatgagagatatctctggcttcatgatgcacaattttaa

SEQ ID NO: 26 - protein, 261 aa, synthetic construct
MGKVFGYPEFDENGEQILTTYDNEYKDMLMDVRVYRMKAGDEKSFQKTGEETAVLLLSGSIEFVFDDVTAKADRKDVFTEGPWCVHAATESKVSVKALADSEILVQSTKNDTKFDTKLYKPEDAPWGYSSVGKFGNVAKRRVNTIFDHDIAPYSNMVLGEVLNDRGNWSGYLPHRHPQPETYYFKFDRPEGFGASFVGDQVFKSTDGSFSAIPGGELHPQAVAPGFQMYTCWMIRHLDGNPWLQTDRNEDERYLWLHDAQF

SEQ ID NO: 27 - DNA, 873 bp, synthetic construct
  source 1..873: mol_type = other DNA
atggcattagtttctgcgacgtcattagtggcaccggcattggcagatcgttacgcaattggtcatttcaatattaatggtgctgattggttagagacgtatctgaaagttgcacaaacgactaagacaccgatcattgtcgccacttccgatcgtatcattgactttctaggcggctttgactatatggctcgctacgtacggtttatgatgcaagcgctcagtgtgacagtaccagttgctttgcatttggaccatgggttatcagttgaccatgtttatcaagcgattgatgctggttacacgtcggtgatgtttgatggttcaaagttgcccattggcgaaaatgtggccttaactaaagaagtcgtagcatatgcccatgcacatcatgtttctgtcgaggccgaagttggtagcgtaggtggtaatgagaatggactcgtcaatgggattcgatatgcaagcgttgctgacgctgttgagatggcttcaacaggtattgacgcattagccgcggcacttggatccgttcacggtgattacgtcggtcggccaaatctgaattttgaacgcatggccgagattgcagcggctactaaattacctttagtgcttcatggtgcgtctggcattttagatgatcagatccaacaggcgattcagttaggcactgcaaaaatcaatatcaatacagaagttaatacagtttggacgagtgctgtgaccaaagccctgcaagccaaacgttccaatcatgacccgcaaccaattttaactgctggtaagcaagcaatcgcgtatttggtagaagcgaagatgaaggcatttcatgtgttagggaaaagtactcgcctatcttctatgagttga

SEQ ID NO: 28 - protein, 290 aa, synthetic construct
MALVSATSLVAPALADRYAIGHFNINGADWLETYLKVAQTTKTPIIVATSDRIIDFLGGFDYMARYVRFMMQALSVTVPVALHLDHGLSVDHVYQAIDAGYTSVMFDGSKLPIGENVALTKEVVAYAHAHHVSVEAEVGSVGGNENGLVNGIRYASVADAVEMASTGIDALAAALGSVHGDYVGRPNLNFERMAEIAAATKLPLVLHGASGILDDQIQQAIQLGTAKININTEVNTVWTSAVTKALQAKRSNHDPQPILTAGKQAIAYLVEAKMKAFHVLGKSTRLSSMS